European Patent Application EP 4 600 364 A1, published August 13, 2025. Title: A novel polynucleotide and method for producing L-alanine using thereof. Applicant: CJ CheilJedang Corporation. Application KR. The sequence listing filed with the application follows.

SEQUENCE LISTING (8 sequences)

SEQ ID NO: 1 - DNA, 100 bp, synthetic construct
  misc_feature 1..100: note = alaT promoter mutantfragment of Corynebacterium glutamicum(100bp)
  source 1..100: mol_type = other DNA
gatcttaggcagccgtgggattacacccttttagagttagaacagtaaaaattcgcccaatagctttcaactacgcacacaaagtggtataattgagcgg

SEQ ID NO: 2 - DNA, 100 bp, synthetic construct
  misc_feature 1..100: note = alaT promoter wild-type fragment of Corynebacterium glutamicum(100bp)
  source 1..100: mol_type = other DNA
gatcttaggcagccgtgggattacacccttttagagttagaacagtaaaaattcgcccaatagctttcaactacgcacacaaagtggcaacattgagcgg

SEQ ID NO: 3 - DNA, 36 bp, synthetic construct
  misc_feature 1..36: note = primer_alaT_AF
  source 1..36: mol_type = other DNA
ctcggtacccggggatccacagcctggtcgcagtcc

SEQ ID NO: 4 - DNA, 36 bp, synthetic construct
  misc_feature 1..36: note = primer_alaT_AR
  source 1..36: mol_type = other DNA
gtctgtagtcatccgctcaattttgccactttgtgt

SEQ ID NO: 5 - DNA, 37 bp, synthetic construct
  misc_feature 1..37: note = primer_alaT_BF
  source 1..37: mol_type = other DNA
acacaaagtggcaaaattgagcggatgactacagaca

SEQ ID NO: 6 - DNA, 36 bp, synthetic construct
  misc_feature 1..36: note = primer_alaT_BR
  source 1..36: mol_type = other DNA
gcatgcctgcaggtcgacgttggcgatcatgtcacg

SEQ ID NO: 7 - DNA, 19 bp, synthetic construct
  misc_feature 1..19: note = primer_alaT_CF
  source 1..19: mol_type = other DNA
acgtcaaagcctgtgcatc

SEQ ID NO: 8 - DNA, 21 bp, synthetic construct
  misc_feature 1..21: note = primer_alaT_CR
  source 1..21: mol_type = other DNA
cagcacgtccttcatcttctc